European Patent Specification EP 2 953 971 B1, published March 1, 2023. Title: IL-11R BINDING PROTEINS AND USES THEREOF. Applicant: CSL Limited. Application EP14749445.4. The sequence listing filed with the application follows.

SEQUENCE LISTING (110 sequences)

SEQ ID NO: 1 - protein, 422 aa, Homo sapiens
MSSSCSGLSRVLVAVATALVSASSPCPQAWGPPGVQYGQPGRSVKLCCPGVTAGDPVSWFRDGEPKLLQGPDSGLGHELVLAQADSTDEGTYICQTLDGALGGTVTLQLGYPPARPVVSCQAADYENFSCTWSPSQISGLPTRYLTSYRKKTVLGADSQRRSPSTGPWPCPQDPLGAARCVVHGAEFWSQYRINVTEVNPLGASTRLLDVSLQSILRPDPPQGLRVESVPGYPRRLRASWTYPASWPCQPHFLLKFRLQYRPAQHPAWSTVEPAGLEEVITDAVAGLPHAVRVSARDFLDAGTWSTWSPEAWGTPSTGTIPKEIPAWGQLHTQPEVEPQVDSPAPPRPSLQPHPRLLDHRDSVEQVAVLASLGILSFLGLVAGALALGLWLRLRRGGKDGSPKPGFLASVIPVDRRPGAPNL

SEQ ID NO: 2 - protein, 432 aa, Macaca fascicularis
MSSSCSGLTRVLVAVATALVSSSSPCPQAWGPPGVQYGQPGRPVMLCCPGVSAGTPVSWFRDGDSRLLQGPDSGLGHRLVLAQVDSPDEGTYVCQTLDGVSGGMVTLKLGFPPARPEVSCQAVDYENFSCTWSPGQVSGLPTRYLTSYRKKTLPGAESQRESPSTGPWPCPQDPLEASRCVVHGAEFWSEYRINVTEVNPLGASTCLLDVRLQSILRPDPPQGLRVESVPGYPRRLHASWTYPASWRRQPHFLLKFRLQYRPAQHPAWSTVEPIGLEEVITDTVAGLPHAVRVSARDFLDAGTWSAWSPEAWGTPSTGLLQDEIPDWSQGHGQQLEAVVAQEDSLAPARPSLQPDPRPLDHRDPLEQVAVLASLGIFSCLGLAVGALALGLWLRLRRSGKEGPQKPGLLAPMIPVEKLPGIPNLQRTPENFS

SEQ ID NO: 3 - protein, 349 aa, artificial
  polypeptide comprising amino acids 23 to 363 of SEQ ID NO: 1 comprising a 8xHIS tag and a serine at a position corresponding to position 248 of SEQ ID NO: 1 (also referred to as "WT F/L")
SSPCPQAWGPPGVQYGQPGRSVKLCCPGVTAGDPVSWFRDGEPKLLQGPDSGLGHELVLAQADSTDEGTYICQTLDGALGGTVTLQLGYPPARPVVSCQAADYENFSCTWSPSQISGLPTRYLTSYRKKTVLGADSQRRSPSTGPWPCPQDPLGAARCVVHGAEFWSQYRINVTEVNPLGASTRLLDVSLQSILRPDPPQGLRVESVPGYPRRLRASWTYPASWPSQPHFLLKFRLQYRPAQHPAWSTVEPAGLEEVITDAVAGLPHAVRVSARDFLDAGTWSTWSPEAWGTPSTGTIPKEIPAWGQLHTQPEVEPQVDSPAPPRPSLQPHPRLLDHRDSVHHHHHHHH

SEQ ID NO: 4 - protein, 422 aa, Homo sapiens; identical to SEQ ID NO: 1

SEQ ID NO: 5 - protein, 107 aa, Artificial Sequence
  amino acid sequence of VL chain of antibody 8E2
DIQMTQSPSSLSASVGDRVTITCQASQDINNYLNWYQQKPGKAPKLLIYDASNLQTGVPSRFSGSGSGTDFTFTISSLQPEDIATYYCQQYDNLSPTFGPGTKVDIK

SEQ ID NO: 6 - protein, 107 aa, Artificial Sequence
  amino acid sequence of VL chain of antibody TS-303
DIQMTQSPSSLSASVGDRVTITCQASQDVDYWVEWYQQKPGKAPKLLIYDASNLQTGVPSRFSGSGSGTDFTFTISSLQPEDIATYYCQQYDNLSPTFGPGTKVDIK

SEQ ID NO: 7 - protein, 107 aa, Artificial Sequence
  amino acid sequence of VL chain of antibody TS-305
DIQMTQSPSSLSASVGDRVTITCQASQDVGIYVEWYQQKPGKAPKLLIYDASNLQTGVPSRFSGSGSGTDFTFTISSLQPEDIATYYCQQYDNLSPTFGPGTKVDIK

SEQ ID NO: 8 - protein, 107 aa, Artificial Sequence
  mino acid sequence of VL chain of antibody TS-306
DIQMTQSPSSLSASVGDRVTITCQASQDVDKYVEWYQQKPGKAPKLLIYDASNLQTGVPSRFSGSGSGTDFTFTISSLQPEDIATYYCQQYDNLSPTFGPGTKVDIK

SEQ ID NO: 9 - protein, 107 aa, Artificial Sequence
  amino acid sequence of VL chain of antibody TS-307
DIQMTQSPSSLSASVGDRVTITCQASQDVSMYVEWYQQKPGKAPKLLIYDASNLQTGVPSRFSGSGSGTDFTFTISSLQPEDIATYYCQQYDNLSPTFGPGTKVDIK

SEQ ID NO: 10 - protein, 107 aa, Artificial Sequence
  amino acid sequence of VL chain of antibody TS-310
DIQMTQSPSSLSASVGDRVTITCQASQDVAMYIEWYQQKPGKAPKLLIYDASNLQTGVPSRFSGSGSGTDFTFTISSLQPEDIATYYCQQYDNLSPTFGPGTKVDIK

SEQ ID NO: 11 - protein, 107 aa, Artificial Sequence
  amino acid sequence of VL chain of antibody TS-311
DIQMTQSPSSLSASVGDRVTITCQASQDVSQYIEWYQQKPGKAPKLLIYDASNLQTGVPSRFSGSGSGTDFTFTISSLQPEDIATYYCQQYDNLSPTFGPGTKVDIK

SEQ ID NO: 12 - protein, 107 aa, Artificial Sequence
  amino acid sequence of VL chain of antibody TS-312
DIQMTQSPSSLSASVGDRVTITCQASQDIGQYVEWYQQKPGKAPKLLIYDASNLQTGVPSRFSGSGSGTDFTFTISSLQPEDIATYYCQQYDNLSPTFGPGTKVDIK

SEQ ID NO: 13 - protein, 107 aa, Artificial Sequence
  amino acid sequence of VL chain of antibody TS-313
DIQMTQSPSSLSASVGDRVTITCQASQDVSGYVEWYQQKPGKAPKLLIYDASNLQTGVPSRFSGSGSGTDFTFTISSLQPEDIATYYCQQYDNLSPTFGPGTKVDIK

SEQ ID NO: 14 - protein, 107 aa, Artificial Sequence
  amino acid sequence of VL chain of antibody TS-322
DIQMTQSPSSLSASVGDRVTITCQASQDVHHYMEWYQQKPGKAPKLLIYDASNLQTGVPSRFSGSGSGTDFTFTISSLQPEDIATYYCQQYDNLSPTFGPGTKVDIK

SEQ ID NO: 15 - protein, 107 aa, Artificial Sequence
  amino acid sequence of VL chain of antibody TS-2
DIQMTQSPSSLSASVGDRVTITCQASQDINNYLNWYQQKPGKAPKLLIYDASNLQTGVPSRFSGSGSGTDFTFTISSLQPEDIATYYCQQAEDQSPTFGPGTKVDIK

SEQ ID NO: 16 - protein, 107 aa, Artificial Sequence
  amino acid sequence of VL chain of antibody TS-4
DIQMTQSPSSLSASVGDRVTITCQASQDINNYLNWYQQKPGKAPKLLIYDASNLQTGVPSRFSGSGSGTDFTFTISSLQPEDIATYYCQQHEFQSPTFGPGTKVDIK

SEQ ID NO: 17 - protein, 107 aa, Artificial Sequence
  amino acid sequence of VL chain of antibody TS-6
DIQMTQSPSSLSASVGDRVTITCQASQDINNYLNWYQQKPGKAPKLLIYDASNLQTGVPSRFSGSGSGTDFTFTISSLQPEDIATYYCEQFESQSPTFGPGTKVDIK

SEQ ID NO: 18 - protein, 107 aa, Artificial Sequence
  amino acid sequence of VL chain of antibody TS-7
DIQMTQSPSSLSASVGDRVTITCQASQDINNYLNWYQQKPGKAPKLLIYDASNLQTGVPSRFSGSGSGTDFTFTISSLQPEDIATYYCQQHENQSPTFGPGTKVDIK

SEQ ID NO: 19 - protein, 107 aa, Artificial Sequence
  amino acid sequence of VL chain of antibody TS-9
DIQMTQSPSSLSASVGDRVTITCQASQDINNYLNWYQQKPGKAPKLLIYDASNLQTGVPSRFSGSGSGTDFTFTISSLQPEDIATYYCQQAEEQSPTFGPGTKVDIK

SEQ ID NO: 20 - protein, 107 aa, Artificial Sequence
  amino acid sequence of VL chain of antibody TS-13
DIQMTQSPSSLSASVGDRVTITCQASQDINNYLNWYQQKPGKAPKLLIYDASNLQTGVPSRFSGSGSGTDFTFTISSLQPEDIATYYCQQNETQSPTFGPGTKVDIK

SEQ ID NO: 21 - protein, 107 aa, Artificial Sequence
  amino acid sequence of VL chain of antibody TS-14
DIQMTQSPSSLSASVGDRVTITCQASQDINNYLNWYQQKPGKAPKLLIYDASNLQTGVPSRFSGSGSGTDFTFTISSLQPEDIATYYCQQHDNQSPTFGPGTKVDIK

SEQ ID NO: 22 - protein, 107 aa, Artificial Sequence
  amino acid sequence of VL chain of antibody TS-17
DIQMTQSPSSLSASVGDRVTITCQASQDINNYLNWYQQKPGKAPKLLIYDASNLQTGVPSRFSGSGSGTDFTFTISSLQPEDIATYYCSQFESQSPTFGPGTKVDIK

SEQ ID NO: 23 - protein, 107 aa, Artificial Sequence
  amino acid sequence of VL chain of antibody TS-20
DIQMTQSPSSLSASVGDRVTITCQASQDINNYLNWYQQKPGKAPKLLIYDASNLQTGVPSRFSGSGSGTDFTFTISSLQPEDIATYYCQQNESQSPTFGPGTKVDIK

SEQ ID NO: 24 - protein, 107 aa, Artificial Sequence
  amino acid sequence of VL chain of antibody TS-21
DIQMTQSPSSLSASVGDRVTITCQASQDINNYLNWYQQKPGKAPKLLIYDASNLQTGVPSRFSGSGSGTDFTFTISSLQPEDIATYYCQQSESQSPTFGPGTKVDIK

SEQ ID NO: 25 - protein, 107 aa, Artificial Sequence
  amino acid sequence of VL chain of antibody TS-22
DIQMTQSPSSLSASVGDRVTITCQASQDINNYLNWYQQKPGKAPKLLIYDASNLQTGVPSRFSGSGSGTDFTFTISSLQPEDIATYYCQQFETQSPTFGPGTKVDIK

SEQ ID NO: 26 - protein, 107 aa, Artificial Sequence
  amino acid sequence of VL chain of antibody TS-29
DIQMTQSPSSLSASVGDRVTITCQASQDINNYLNWYQQKPGKAPKLLIYDASNLQTGVPSRFSGSGSGTDFTFTISSLQPEDIATYYCQQSEEQSPTFGPGTKVDIK

SEQ ID NO: 27 - protein, 107 aa, Artificial Sequence
  amino acid sequence of VL chain of antibody TS-32
DIQMTQSPSSLSASVGDRVTITCQASQDINNYLNWYQQKPGKAPKLLIYDASNLQTGVPSRFSGSGSGTDFTFTISSLQPEDIATYYCTQWETQSPTFGPGTKVDIK

SEQ ID NO: 28 - protein, 107 aa, Artificial Sequence
  amino acid sequence of VL chain of antibody TS-49
DIQMTQSPSSLSASVGDRVTITCQASQDINNYLNWYQQKPGKAPKLLIYDASNLQTGVPSRFSGSGSGTDFTFTISSLQPEDIATYYCQQYESQAPEFGPGTKVDIK

SEQ ID NO: 29 - protein, 107 aa, Artificial Sequence
  amino acid sequence of VL chain of antibody TS-51
DIQMTQSPSSLSASVGDRVTITCQASQDINNYLNWYQQKPGKAPKLLIYDASNLQTGVPSRFSGSGSGTDFTFTISSLQPEDIATYYCQQYESQWPFFGPGTKVDIK

SEQ ID NO: 30 - protein, 107 aa, Artificial Sequence
  amino acid sequence of VL chain of antibody TS-55
DIQMTQSPSSLSASVGDRVTITCQASQDINNYLNWYQQKPGKAPKLLIYDASNLQTGVPSRFSGSGSGTDFTFTISSLQPEDIATYYCQQYETQTPAFGPGTKVDIK

SEQ ID NO: 31 - protein, 107 aa, Artificial Sequence
  amino acid sequence of VL chain of antibody TS-57
DIQMTQSPSSLSASVGDRVTITCQASQDINNYLNWYQQKPGKAPKLLIYDASNLQTGVPSRFSGSGSGTDFTFTISSLQPEDIATYYCQQYETQMPLFGPGTKVDIK

SEQ ID NO: 32 - protein, 107 aa, Artificial Sequence
  amino acid sequence of VL chain of antibody TS-58
DIQMTQSPSSLSASVGDRVTITCQASQDINNYLNWYQQKPGKAPKLLIYDASNLQTGVPSRFSGSGSGTDFTFTISSLQPEDIATYYCQQYETQQPFFGPGTKVDIK

SEQ ID NO: 33 - protein, 107 aa, Artificial Sequence
  amino acid sequence of VL chain of antibody TS-63
DIQMTQSPSSLSASVGDRVTITCQASQDINNYLNWYQQKPGKAPKLLIYDASNLQTGVPSRFSGSGSGTDFTFTISSLQPEDIATYYCQQYDTQQPNFGPGTKVDIK

SEQ ID NO: 34 - protein, 107 aa, Artificial Sequence
  amino acid sequence of VL chain of antibody TS-64
DIQMTQSPSSLSASVGDRVTITCQASQDINNYLNWYQQKPGKAPKLLIYDASNLQTGVPSRFSGSGSGTDFTFTISSLQPEDIATYYCQQYESQWPQFGPGTKVDIK

SEQ ID NO: 35 - protein, 107 aa, Artificial Sequence
  amino acid sequence of consensus of VL chain of 8E2 antibody and derivatives
  VARIANT (29)..(29): X=I or V
  VARIANT (30)..(30): X=N or D or G or S or A or H
  VARIANT (31)..(31): X=N or Y or I or K or M or Q or G or H
  VARIANT (32)..(32): X=Y or W
  VARIANT (33)..(33): X=L or V or I or M
  VARIANT (34)..(34): X=N or E
  VARIANT (89)..(89): X=Q or E or S or T
  VARIANT (91)..(91): X=Y or A or H or F or N or S or W
  VARIANT (92)..(92): X=D or E
  VARIANT (93)..(93): X=N or D or F or S or E or T
  VARIANT (94)..(94): X=L or Q
  VARIANT (95)..(95): X=S or A or W or T or M or Q
  VARIANT (97)..(97): X=T or E or F or A or L or N or Q
DIQMTQSPSSLSASVGDRVTITCQASQDXXXXXXWYQQKPGKAPKLLIYDASNLQTGVPSRFSGSGSGTDFTFTISSLQPEDIATYYCXQXXXXXPXFGPGTKVDIK

SEQ ID NO: 36 - protein, 107 aa, Artificial Sequence
  amino acid sequence of consensus of VL chain of 8E2 antibody and select derivatives
  VARIANT (29)..(29): X=I or V
  VARIANT (30)..(30): X=D or N
  VARIANT (31)..(31): X=K or N
  VARIANT (33)..(33): X=L or V
  VARIANT (34)..(34): X=N or E
  VARIANT (91)..(91): X=Y or A or H
  VARIANT (92)..(92): X=D or E
  VARIANT (93)..(93): X=N or D or F or N or S
  VARIANT (94)..(94): X=L or Q
  VARIANT (95)..(95): X=S or W
  VARIANT (97)..(97): X=T or F
DIQMTQSPSSLSASVGDRVTITCQASQDXXXYXXWYQQKPGKAPKLLIYDASNLQTGVPSRFSGSGSGTDFTFTISSLQPEDIATYYCQQXXXXXPXFGPGTKVDIK

SEQ ID NO: 37 - protein, 118 aa, Artificial Sequence
  amino acid sequence of VH chain of antibody 8E2
EVQLLESGGGLVQPGGSLRLSCAASGFTFSWYSMTWVRQAPGKGLEWVSSIVPSGGHTQYADSVKGRFTISRDNSKNTLYLQMNSLRAEDTAVYYCAKGPGWGSFDLWGRGTLVTVSS

SEQ ID NO: 38 - protein, 118 aa, Artificial Sequence
  amino acid sequence of VH chain of antibody TS-66
EVQLLESGGGLVQPGGSLRLSCAASGFTFAWWSIAWVRQAPGKGLEWVSSIVPSGGHTQYADSVKGRFTISRDNSKNTLYLQMNSLRAEDTAVYYCAKGPGWGSFDLWGRGTLVTVSS

SEQ ID NO: 39 - protein, 118 aa, Artificial Sequence
  amino acid sequence of VH chain of antibody TS-69
EVQLLESGGGLVQPGGSLRLSCAASGFTFGWWSVTWVRQAPGKGLEWVSSIVPSGGHTQYADSVKGRFTISRDNSKNTLYLQMNSLRAEDTAVYYCAKGPGWGSFDLWGRGTLVTVSS

SEQ ID NO: 40 - protein, 118 aa, Artificial Sequence
  amino acid sequence of VH chain of antibody TS-71
EVQLLESGGGLVQPGGSLRLSCAASGFTFWRWSTTWVRQAPGKGLEWVSSIVPSGGHTQYADSVKGRFTISRDNSKNTLYLQMNSLRAEDTAVYYCAKGPGWGSFDLWGRGTLVTVSS

SEQ ID NO: 41 - protein, 118 aa, Artificial Sequence
  amino acid sequence of VH chain of antibody TS-76
EVQLLESGGGLVQPGGSLRLSCAASGFTFWRWSITWVRQAPGKGLEWVSSIVPSGGHTQYADSVKGRFTISRDNSKNTLYLQMNSLRAEDTAVYYCAKGPGWGSFDLWGRGTLVTVSS

SEQ ID NO: 42 - protein, 118 aa, Artificial Sequence
  amino acid sequence of VH chain of antibody TS-79
EVQLLESGGGLVQPGGSLRLSCAASGFTFAWFSVTWVRQAPGKGLEWVSSIVPSGGHTQYADSVKGRFTISRDNSKNTLYLQMNSLRAEDTAVYYCAKGPGWGSFDLWGRGTLVTVSS

SEQ ID NO: 43 - protein, 118 aa, Artificial Sequence
  amino acid sequence of VH chain of antibody TS-82
EVQLLESGGGLVQPGGSLRLSCAASGFTFWRWSVTWVRQAPGKGLEWVSSIVPSGGHTQYADSVKGRFTISRDNSKNTLYLQMNSLRAEDTAVYYCAKGPGWGSFDLWGRGTLVTVSS

SEQ ID NO: 44 - protein, 118 aa, Artificial Sequence; identical to SEQ ID NO: 40
  amino acid sequence of VH chain of antibody TS-88

SEQ ID NO: 45 - protein, 118 aa, Artificial Sequence; identical to SEQ ID NO: 41
  amino acid sequence of VH chain of antibody TS-89

SEQ ID NO: 46 - protein, 118 aa, Artificial Sequence
  amino acid sequence of VH chain of antibody TS-91
EVQLLESGGGLVQPGGSLRLSCAASGFTFGWWSLTWVRQAPGKGLEWVSSIVPSGGHTQYADSVKGRFTISRDNSKNTLYLQMNSLRAEDTAVYYCAKGPGWGSFDLWGRGTLVTVSS

SEQ ID NO: 47 - protein, 118 aa, Artificial Sequence
  amino acid sequence of VH chain of antibody TS-92
EVQLLESGGGLVQPGGSLRLSCAASGFTFSWWSITWVRQAPGKGLEWVSSIVPSGGHTQYADSVKGRFTISRDNSKNTLYLQMNSLRAEDTAVYYCAKGPGWGSFDLWGRGTLVTVSS

SEQ ID NO: 48 - protein, 118 aa, Artificial Sequence
  amino acid sequence of VH chain of antibody TS-97
EVQLLESGGGLVQPGGSLRLSCAASGFTFSWYSMTWVRQAPGKGLEWVSSIVPWADYTQYADSVKGRFTISRDNSKNTLYLQMNSLRAEDTAVYYCAKGPGWGSFDLWGRGTLVTVSS

SEQ ID NO: 49 - protein, 118 aa, Artificial Sequence
  amino acid sequence of VH chain of antibody TS-101
EVQLLESGGGLVQPGGSLRLSCAASGFTFSWYSMTWVRQAPGKGLEWVSSIVPWGDLTQYADSVKGRFTISRDNSKNTLYLQMNSLRAEDTAVYYCAKGPGWGSFDLWGRGTLVTVSS

SEQ ID NO: 50 - protein, 118 aa, Artificial Sequence
  amino acid sequence of VH chain of antibody TS-103
EVQLLESGGGLVQPGGSLRLSCAASGFTFSWYSMTWVRQAPGKGLEWVSSIVPYGDLTQYADSVKGRFTISRDNSKNTLYLQMNSLRAEDTAVYYCAKGPGWGSFDLWGRGTLVTVSS

SEQ ID NO: 51 - protein, 118 aa, Artificial Sequence
  amino acid sequence of VH chain of antibody TS-104
EVQLLESGGGLVQPGGSLRLSCAASGFTFSWYSMTWVRQAPGKGLEWVSSIVPWGTITQYADSVKGRFTISRDNSKNTLYLQMNSLRAEDTAVYYCAKGPGWGSFDLWGRGTLVTVSS

SEQ ID NO: 52 - protein, 118 aa, Artificial Sequence
  amino acid sequence of VH chain of antibody TS-107
EVQLLESGGGLVQPGGSLRLSCAASGFTFSWYSMTWVRQAPGKGLEWVSSIVPWGDFTQYADSVKGRFTISRDNSKNTLYLQMNSLRAEDTAVYYCAKGPGWGSFDLWGRGTLVTVSS

SEQ ID NO: 53 - protein, 118 aa, Artificial Sequence
  amino acid sequence of VH chain of antibody TS-108
EVQLLESGGGLVQPGGSLRLSCAASGFTFSWYSMTWVRQAPGKGLEWVSSIVPWGTLTQYADSVKGRFTISRDNSKNTLYLQMNSLRAEDTAVYYCAKGPGWGSFDLWGRGTLVTVSS

SEQ ID NO: 54 - protein, 118 aa, Artificial Sequence
  amino acid sequence of VH chain of antibody TS-115
EVQLLESGGGLVQPGGSLRLSCAASGFTFSWYSMTWVRQAPGKGLEWVSSIVPHGDLTQYADSVKGRFTISRDNSKNTLYLQMNSLRAEDTAVYYCAKGPGWGSFDLWGRGTLVTVSS

SEQ ID NO: 55 - protein, 118 aa, Artificial Sequence
  amino acid sequence of VH chain of antibody TS-129
EVQLLESGGGLVQPGGSLRLSCAASGFTFSWYSMTWVRQAPGKGLEWVSSIVPSGGHTQYADSVKGRFTISRDNSKNTLYLQMNSLRAEDTAVYYCAKPEDWGMFDLWGRGTLVTVSS

SEQ ID NO: 56 - protein, 118 aa, Artificial Sequence
  amino acid sequence of VH chain of antibody TS-133
EVQLLESGGGLVQPGGSLRLSCAASGFTFSWYSMTWVRQAPGKGLEWVSSIVPSGGHTQYADSVKGRFTISRDNSKNTLYLQMNSLRAEDTAVYYCAKPVDWGRFDLWGRGTLVTVSS

SEQ ID NO: 57 - protein, 118 aa, Artificial Sequence
  amino acid sequence of VH chain of antibody TS-134
EVQLLESGGGLVQPGGSLRLSCAASGFTFSWYSMTWVRQAPGKGLEWVSSIVPSGGHTQYADSVKGRFTISRDNSKNTLYLQMNSLRAEDTAVYYCAKPEDWGLFDLWGRGTLVTVSS

SEQ ID NO: 58 - protein, 118 aa, Artificial Sequence
  amino acid sequence of VH chain of antibody TS-135
EVQLLESGGGLVQPGGSLRLSCAASGFTFSWYSMTWVRQAPGKGLEWVSSIVPSGGHTQYADSVKGRFTISRDNSKNTLYLQMNSLRAEDTAVYYCAKPLDWGLFDLWGRGTLVTVSS

SEQ ID NO: 59 - protein, 118 aa, Artificial Sequence
  amino acid sequence of VH chain of antibody TS-136
EVQLLESGGGLVQPGGSLRLSCAASGFTFSWYSMTWVRQAPGKGLEWVSSIVPSGGHTQYADSVKGRFTISRDNSKNTLYLQMNSLRAEDTAVYYCAKPLDWGRFDLWGRGTLVTVSS

SEQ ID NO: 60 - protein, 118 aa, Artificial Sequence
  amino acid sequence of VH chain of antibody TS-140
EVQLLESGGGLVQPGGSLRLSCAASGFTFSWYSMTWVRQAPGKGLEWVSSIVPSGGHTQYADSVKGRFTISRDNSKNTLYLQMNSLRAEDTAVYYCAKPNDWGLFDLWGRGTLVTVSS

SEQ ID NO: 61 - protein, 118 aa, Artificial Sequence
  amino acid sequence of VH chain of antibody TS-143
EVQLLESGGGLVQPGGSLRLSCAASGFTFSWYSMTWVRQAPGKGLEWVSSIVPSGGHTQYADSVKGRFTISRDNSKNTLYLQMNSLRAEDTAVYYCAKPHDWGLFDLWGRGTLVTVSS

SEQ ID NO: 62 - protein, 118 aa, Artificial Sequence
  amino acid sequence of VH chain of antibody TS-151
EVQLLESGGGLVQPGGSLRLSCAASGFTFSWYSMTWVRQAPGKGLEWVSSIVPSGGHTQYADSVKGRFTISRDNSKNTLYLQMNSLRAEDTAVYYCAKPHDWGRFDLWGRGTLVTVSS

SEQ ID NO: 63 - protein, 118 aa, Artificial Sequence
  amino acid sequence of VH chain of antibody TS-156
EVQLLESGGGLVQPGGSLRLSCAASGFTFSWYSMTWVRQAPGKGLEWVSSIVPSGGHTQYADSVKGRFTISRDNSKNTLYLQMNSLRAEDTAVYYCAKPEDWGRFDLWGRGTLVTVSS

SEQ ID NO: 64 - protein, 118 aa, Artificial Sequence
  amino acid sequence of VH chain of antibody TS-213
EVQLLESGGGLVQPGGSLRLSCAASGFTFSWYSMTWVRQAPGKGLEWVSSIVPSGGHTQYADSVKGRFTISRDNSKNTLYLQMNSLRAEDTAVYYCAKGPGWGQFAVWGRGTLVTVSS

SEQ ID NO: 65 - protein, 118 aa, Artificial Sequence
  amino acid sequence of VH chain of antibody TS-214
EVQLLESGGGLVQPGGSLRLSCAASGFTFSWYSMTWVRQAPGKGLEWVSSIVPSGGHTQYADSVKGRFTISRDNSKNTLYLQMNSLRAEDTAVYYCAKGPGWGSFWFWGRGTLVTVSS

SEQ ID NO: 66 - protein, 118 aa, Artificial Sequence
  amino acid sequence of VH chain of antibody TS-215
EVQLLESGGGLVQPGGSLRLSCAASGFTFSWYSMTWVRQAPGKGLEWVSSIVPSGGHTQYADSVKGRFTISRDNSKNTLYLQMNSLRAEDTAVYYCAKGPGWGSFWQWGRGTLVTVSS

SEQ ID NO: 67 - protein, 118 aa, Artificial Sequence
  amino acid sequence of VH chain of antibody TS-218
EVQLLESGGGLVQPGGSLRLSCAASGFTFSWYSMTWVRQAPGKGLEWVSSIVPSGGHTQYADSVKGRFTISRDNSKNTLYLQMNSLRAEDTAVYYCAKGPGWGSFWEWGRGTLVTVSS

SEQ ID NO: 68 - protein, 118 aa, Artificial Sequence
  amino acid sequence of VH chain of antibody TS-221
EVQLLESGGGLVQPGGSLRLSCAASGFTFSWYSMTWVRQAPGKGLEWVSSIVPSGGHTQYADSVKGRFTISRDNSKNTLYLQMNSLRAEDTAVYYCAKGPGWGSFWYWGRGTLVTVSS

SEQ ID NO: 69 - protein, 118 aa, Artificial Sequence
  amino acid sequence of VH chain of antibody TS-222
EVQLLESGGGLVQPGGSLRLSCAASGFTFSWYSMTWVRQAPGKGLEWVSSIVPSGGHTQYADSVKGRFTISRDNSKNTLYLQMNSLRAEDTAVYYCAKGPGWGTFAYWGRGTLVTVSS

SEQ ID NO: 70 - protein, 118 aa, Artificial Sequence
  amino acid sequence of VH chain of antibody TS-224
EVQLLESGGGLVQPGGSLRLSCAASGFTFSWYSMTWVRQAPGKGLEWVSSIVPSGGHTQYADSVKGRFTISRDNSKNTLYLQMNSLRAEDTAVYYCAKGPGWGSFWTWGRGTLVTVSS

SEQ ID NO: 71 - protein, 118 aa, Artificial Sequence
  amino acid sequence of consensus of VH chain of 8E2 antibody and derivatives
  misc_feature (30)..(30): Xaa can be any naturally occurring amino acid
  VARIANT (31)..(31): X=W or R
  VARIANT (32)..(32): X=Y or W or F
  VARIANT (34)..(34): X=M or I or V or T or L
  VARIANT (35)..(35): X=T or A
  VARIANT (54)..(54): X=S or W or Y or H
  VARIANT (55)..(55): X=G or A
  VARIANT (56)..(56): X=G or D or T
  VARIANT (57)..(57): X=H or Y or L or I or F
  VARIANT (99)..(99): X=G or P
  VARIANT (100)..(100): X=P or E or V or L or N or H or E
  VARIANT (101)..(101): X=G or D
  VARIANT (104)..(104): X=S or M or R or L or Q or T
  VARIANT (106)..(106): X=D or A or W
  VARIANT (107)..(107): X=L or V or F or Q or E or Y or T
EVQLLESGGGLVQPGGSLRLSCAASGFTFXXXSXXWVRQAPGKGLEWVSSIVPXXXXTQYADSVKGRFTISRDNSKNTLYLQMNSLRAEDTAVYYCAKXXXWGXFXXWGRGTLVTVSS

SEQ ID NO: 72 - protein, 118 aa, Artificial Sequence
  amino acid sequence of consensus of VH chain of 8E2 antibody and select derivatives
  VARIANT (54)..(54): X=W or S
  VARIANT (56)..(56): X=G or D or T
  VARIANT (57)..(57): X=H or L
  VARIANT (99)..(99): X=G or P
  VARIANT (100)..(100): X=P or E or L
  VARIANT (101)..(101): X=G or D
  VARIANT (104)..(104): X=S or L or R
EVQLLESGGGLVQPGGSLRLSCAASGFTFSWYSMTWVRQAPGKGLEWVSSIVPXGXXTQYADSVKGRFTISRDNSKNTLYLQMNSLRAEDTAVYYCAKXXXWGXFDLWGRGTLVTVSS

SEQ ID NO: 73 - protein, 114 aa, Artificial Sequence
  amino acid sequence of VL chain of antibody 8E4
QSALTQPPSASGSPGQSVAISCTGTSSDVGGYNFVSWYQQHPGKAPKLLIYEVTKRPSGVPDRFSGSKAGNTASLTVSGLQAEDEADYYCSSYGGSNNAGVFGTGTKVTVLGQP

SEQ ID NO: 74 - protein, 126 aa, Artificial Sequence
  amino acid sequence of VH chain of antibody 8E4
EVQLLESGGGLVQPGGSLRLSCAASGFTFSWYFMGWVRQAPGKGLEWVSYIYPSGGSTGYADSVKGRFTISRDNSKNTLYLQMHSLRAEDTAVYYCARDEGYCSSTSCYFDAFDIWGQGTMVTVSS

SEQ ID NO: 75 - protein, 107 aa, Artificial Sequence
  amino acid sequence of VL chain of antibody 8D10
DIQMTQSPSSLSASVGDRVTITCQASQDITNYLNWYLHKPGKAPKLLIYDASNLQTGVPSRFSGSGSGTDFTFTITSLQPEDFGTYYCQQYDTLHPSFGPGTTVDIK

SEQ ID NO: 76 - protein, 118 aa, Artificial Sequence
  amino acid sequence of VH chain of antibody 8D10
EVQLLESGGGLVQPGGSLRLSCAASGFTFSRYMMGWVRQAPGKGLEWVSSIVPSGGITIYADSVKGRFTISRDNSKNTLYLQMNSLRAEDTAVYYCARDHMGIVATDWGQGTLVTVSS

SEQ ID NO: 77 - protein, 11 aa, Artificial Sequence
  amino acid sequence of consensus of CDR1 of VL chain of 8E2 antibody and derivatives
  VARIANT (6)..(6): X=I or V
  VARIANT (7)..(7): X=N or D or G or S or A or H
  VARIANT (8)..(8): X=N or Y or I or K or M or Q or G or H
  VARIANT (9)..(9): X=Y or W
  VARIANT (10)..(10): X=L or V or I or M
  VARIANT (11)..(11): X=N or E
QASQDXXXXXX

SEQ ID NO: 78 - protein, 9 aa, Artificial Sequence
  amino acid sequence of consensus of CDR3 of VL chain of 8E2 antibody and derivatives
  VARIANT (1)..(1): X=Q or E or S or T
  VARIANT (3)..(3): X=Y or A or H or F or N or S or W
  VARIANT (4)..(4): X=D or E
  VARIANT (5)..(5): X=N or D or F or S or E or T
  VARIANT (6)..(6): X=L or Q
  misc_feature (7)..(7): Xaa can be any naturally occurring amino acid
  VARIANT (9)..(9): X=T or F or A or L or N or Q
XQXXXXXPX

SEQ ID NO: 79 - protein, 5 aa, Artificial Sequence
  amino acid sequence of consensus of CDR1 of VH chain of 8E2 antibody and derivatives
  VARIANT (1)..(1): X=W or R
  VARIANT (2)..(2): X=Y or W or F
  VARIANT (4)..(4): X=M or I or V or T or L
  VARIANT (5)..(5): X=T or A
XXSXX

SEQ ID NO: 80 - protein, 17 aa, Artificial Sequence
  amino acid sequence of consensus of CDR2 of VH chain of 8E2 antibody and derivatives
  VARIANT (5)..(5): X=S or W or Y or H
  VARIANT (6)..(6): X=G or A
  VARIANT (7)..(7): X=G or D or T
  VARIANT (8)..(8): X=H or Y or L or I or F
SIVPXXXXTQYADSVKG

SEQ ID NO: 81 - protein, 9 aa, Artificial Sequence
  amino acid sequence of consensus of CDR3 of VH chain of 8E2 antibody and derivatives
  VARIANT (1)..(1): X=G or P
  VARIANT (2)..(2): X=P or E or V or L or N or H or E
  VARIANT (3)..(3): X=G or D
  VARIANT (6)..(6): X=S or M or R or L or Q or T
  VARIANT (8)..(8): X=D or A or W
  VARIANT (9)..(9): X=L or V or F or Q or E or Y or T
XXXWGXFXX

SEQ ID NO: 82 - protein, 424 aa, Mus musculus
MSSSCSGLTRVLVAVATALVSSSSPCPQAWGPPGVQYGQPGRPVMLCCPGVSAGTPVSWFRDGDSRLLQGPDSGLGHRLVLAQVDSPDEGTYVCQTLDGVSGGMVTLKLGFPPARPEVSCQAVDYENFSCTWSPGQVSGLPTRYLTSYRKKTLPGAESQRESPSTGPWPCPQDPLEASRCVVHGAEFWSEYRINVTEVNPLGASTCLLDVRLQSILRPDPPQGLRVESVPGYPRRLHASWTYPASWRRQPHFLLKFRLQYRPAQHPAWSTVEPIGLEEVITDTVAGLPHAVRVSARDFLDAGTWSAWSPEAWGTPSTGLLQDEIPDWSQGHGQQLEAVVAQEDSLAPARPSLQPDPRPLDHRDPLEQVAVLASLGIFSCLGLAVGALALGLWLRLRRSGKEGPQKPGLLAPMIPVEKLPGIPNL

SEQ ID NO: 83 - protein, 214 aa, Artificial Sequence
  amino acid sequence of heavy chain of antibody 8E2
DIQMTQSPSSLSASVGDRVTITCQASQDINNYLNWYQQKPGTAPKLLIYDASNLQTGVPSRFSGSGSGTHFTFTINTLQPEDIATYYCQQYDNLSPTFGPGTKVDIKRTVAAPSVFIFPPSDEQLKSGTASVVCLLNNFYPREAKVQWKVDNALQSGNSQESVTEQDSKDSTYSLSSTLTLSKADYEKHKVYACEVTHQGLSSPVTKSFNRGEC

SEQ ID NO: 84 - protein, 302 aa, Artificial Sequence
  amino acid sequence of light chain of antibody 8E2
EVQLLESGGGLVQPGGSLRLSCAASGFTFSWYSMTWVRQAPGKGLEWVSSIVPSGGHTQYADSVKGRFTISRDNSKNTLYLQMNSLRAEDTAVYYCAKGPGWGSFDLWGRGTLVTVSSASTKGPSVFPLAPCSRSTSESTAALGCLVKDYFPEPVTVSWNSGALTSGVHTFPAVLQSSGLYSLSSVVTVPSSSLGTKTYTCNVDHKPSNTKVDKRVESKYGPPCPPCPAPEFLGGPSVFLFPPKPKDTLMISRTPEVTCVVVDVSQEDPEVQFNWYVDGVEVHNAKTKPREEQFNSTYRVVS

SEQ ID NO: 85 - protein, 304 aa, Artificial Sequence
  polypeptide comprising amino acids 23 to 318 of Homo sapiens IL-11R? (SEQ ID NO: 1), a 8xHIS tag and a serine at a position corresponding to position 248 of SEQ ID NO:1 (also referred to as "WT D1/2")
SSPCPQAWGPPGVQYGQPGRSVKLCCPGVTAGDPVSWFRDGEPKLLQGPDSGLGHELVLAQADSTDEGTYICQTLDGALGGTVTLQLGYPPARPVVSCQAADYENFSCTWSPSQISGLPTRYLTSYRKKTVLGADSQRRSPSTGPWPCPQDPLGAARCVVHGAEFWSQYRINVTEVNPLGASTRLLDVSLQSILRPDPPQGLRVESVPGYPRRLRASWTYPASWPSQPHFLLKFRLQYRPAQHPAWSTVEPAGLEEVITDAVAGLPHAVRVSARDFLDAGTWSTWSPEAWGTPSTGHHHHHHHH

SEQ ID NO: 86 - protein, 353 aa, Artificial Sequence
  amino acid sequence of a polypeptide comprising amino acids 23-110 of SEQ ID NO: 1 and amino acids 111-367 of SEQ ID NO: 82 in which there is a serine at a position corresponding to position 206 of SEQ ID NO: 82 and a HIS tag
SSPCPQAWGPPGVQYGQPGRSVKLCCPGVTAGDPVSWFRDGEPKLLQGPDSGLGHELVLAQADSTDEGTYICQTLDGALGGTVTLQLGFPPARPEVSCQAVDYENFSCTWSPGQVSGLPTRYLTSYRKKTLPGAESQRESPSTGPWPCPQDPLEASRCVVHGAEFWSEYRINVTEVNPLGASTSLLDVRLQSILRPDPPQGLRVESVPGYPRRLHASWTYPASWRRQPHFLLKFRLQYRPAQHPAWSTVEPIGLEEVITDAVAGLPHAVRVSARDFLDAGTWSAWSPEAWGTPSTGPLQDEIPDWSQGHGQQLEAVVAQEDSPAPARPSLQPDPRPLDHRDPLEQHHHHHHHH

SEQ ID NO: 87 - protein, 353 aa, Artificial Sequence
  amino acid sequence of a polypeptide comprising amino acids 23-215 of SEQ ID NO: 1 and amino acids 216-367 of SEQ ID NO: 82 and a HIS tag
SSPCPQAWGPPGVQYGQPGRSVKLCCPGVTAGDPVSWFRDGEPKLLQGPDSGLGHELVLAQADSTDEGTYICQTLDGALGGTVTLQLGYPPARPVVSCQAADYENFSCTWSPSQISGLPTRYLTSYRKKTVLGADSQRRSPSTGPWPCPQDPLGAARCVVHGAEFWSQYRINVTEVNPLGASTRLLDVSLQSILRPDPPQGLRVESVPGYPRRLHASWTYPASWRRQPHFLLKFRLQYRPAQHPAWSTVEPIGLEEVITDAVAGLPHAVRVSARDFLDAGTWSAWSPEAWGTPSTGPLQDEIPDWSQGHGQQLEAVVAQEDSPAPARPSLQPDPRPLDHRDPLEQHHHHHHHH

SEQ ID NO: 88 - protein, 353 aa, Artificial Sequence
  amino acid sequence of a polypeptide comprising amino acids 23-318 of SEQ ID NO: 1 in which there is a serine at a position corresponding to position 226 of SEQ ID NO: 1 and amino acids 319-367 of SEQ ID NO: 82 and a HIS tag
SSPCPQAWGPPGVQYGQPGRSVKLCCPGVTAGDPVSWFRDGEPKLLQGPDSGLGHELVLAQADSTDEGTYICQTLDGALGGTVTLQLGYPPARPVVSCQAADYENFSCTWSPSQISGLPTRYLTSYRKKTVLGADSQRRSPSTGPWPCPQDPLGAARCVVHGAEFWSQYRINVTEVNPLGASTRLLDVSLQSILRPDPPQGLRVESVPGYPRRLRASWTYPASWPSQPHFLLKFRLQYRPAQHPAWSTVEPAGLEEVITDAVAGLPHAVRVSARDFLDAGTWSTWSPEAWGTPSTGPLQDEIPDWSQGHGQQLEAVVAQEDSPAPARPSLQPDPRPLDHRDPLEQHHHHHHHH

SEQ ID NO: 89 - protein, 348 aa, Artificial Sequence
  amino acid sequence of a polypeptide comprising amino acids 24-215 of SEQ ID NO: 82 in which there is a serine at a position corresponding to position 206 of SEQ ID NO: 82 and amino acids 216-363 of SEQ ID NO: 1 and a HIS tag
SPCPQAWGPPGVQYGQPGRPVMLCCPGVSAGTPVSWFRDGDSRLLQGPDSGLGHRLVLAQVDSPDEGTYVCQTLDGVSGGMVTLKLGFPPARPEVSCQAVDYENFSCTWSPGQVSGLPTRYLTSYRKKTLPGAESQRESPSTGPWPCPQDPLEASRCVVHGAEFWSEYRINVTEVNPLGASTSLLDVRLQSILRPDPPQGLRVESVPGYPRRLRASWTYPASWPSQPHFLLKFRLQYRPAQHPAWSTVEPAGLEEVITDAVAGLPHAVRVSARDFLDAGTWSTWSPEAWGTPSTGTIPKEIPAWGQLHTQPEVEPQVDSPAPPRPSLQPHPRLLDHRDSVHHHHHHHH

SEQ ID NO: 90 - protein, 352 aa, artificial
  amino acid sequence of Mus musculus sIL-11Ra comprising amino acids 24 to 367 of SEQ ID NO: 82 comprising a HIS tag and a serine at a position corresponding to position 206 of SEQ ID NO: 82
SPCPQAWGPPGVQYGQPGRPVMLCCPGVSAGTPVSWFRDGDSRLLQGPDSGLGHRLVLAQVDSPDEGTYVCQTLDGVSGGMVTLKLGFPPARPEVSCQAVDYENFSCTWSPGQVSGLPTRYLTSYRKKTLPGAESQRESPSTGPWPCPQDPLEASRCVVHGAEFWSEYRINVTEVNPLGASTSLLDVRLQSILRPDPPQGLRVESVPGYPRRLHASWTYPASWRRQPHFLLKFRLQYRPAQHPAWSTVEPIGLEEVITDAVAGLPHAVRVSARDFLDAGTWSAWSPEAWGTPSTGPLQDEIPDWSQGHGQQLEAVVAQEDSPAPARPSLQPDPRPLDHRDPLEQHHHHHHHH

SEQ ID NO: 91 - protein, 217 aa, Artificial Sequence
  amino acid sequence of light chain of antibody 8E4
QSALTQPPSASGSPGQSVAISCTGTSSDVGGYNFVSWYQQHPGKAPKLLIYEVTKRPSGVPDRFSGSKAGNTASLTVSGLQAEDEADYYCSSYGGSNNAGVFGTGTKVTVLGQPKANPTVTLFPPSSEELQANKATLVCLISDFYPGAVTVAWKADGSPVKAGVETTKPSKQSNNKYAASSYLSLTPEQWKSHRSYSCQVTHEGSTVEKTVAPTECS

SEQ ID NO: 92 - protein, 453 aa, Artificial Sequence
  amino acid sequence of heavy chain of antibody 8E4
EVQLLESGGGLVQPGGSLRLSCAASGFTFSWYFMGWVRQAPGKGLEWVSYIYPSGGSTGYADSVKGRFTISRDNSKNTLYLQMHSLRAEDTAVYYCARDEGYCSSTSCYFDAFDIWGQGTMVTVSSASTKGPSVFPLAPCSRSTSESTAALGCLVKDYFPEPVTVSWNSGALTSGVHTFPAVLQSSGLYSLSSVVTVPSSSLGTKTYTCNVDHKPSNTKVDKRVESKYGPPCPPCPAPEFLGGPSVFLFPPKPKDTLMISRTPEVTCVVVDVSQEDPEVQFNWYVDGVEVHNAKTKPREEQFNSTYRVVSVLTVLHQDWLNGKEYKCKVSNKGLPSSIEKTISKAKGQPREPQVYTLPPSQEEMTKNQVSLTCLVKGFYPSDIAVEWESNGQPENNYKTTPPVLDSDGSFFLYSRLTVDKSRWQEGNVFSCSVMHEALHNHYTQKSLSLSLGK

SEQ ID NO: 93 - protein, 214 aa, Artificial Sequence
  amino acid sequence of light chain of antibody 8D10
DIQMTQSPSSLSASVGDRVTITCQASQDITNYLNWYLHKPGKAPKLLIYDASNLQTGVPSRFSGSGSGTDFTFTITSLQPEDFGTYYCQQYDTLHPSFGPGTTVDIKRTVAAPSVFIFPPSDEQLKSGTASVVCLLNNFYPREAKVQWKVDNALQSGNSQESVTEQDSKDSTYSLSSTLTLSKADYEKHKVYACEVTHQGLSSPVTKSFNRGEC

SEQ ID NO: 94 - protein, 445 aa, Artificial Sequence
  amino acid sequence of heavy chain of antibody 8D10
EVQLLESGGGLVQPGGSLRLSCAASGFTFSRYMMGWVRQAPGKGLEWVSSIVPSGGITIYADSVKGRFTISRDNSKNTLYLQMNSLRAEDTAVYYCARDHMGIVATDWGQGTLVTVSSASTKGPSVFPLAPCSRSTSESTAALGCLVKDYFPEPVTVSWNSGALTSGVHTFPAVLQSSGLYSLSSVVTVPSSSLGTKTYTCNVDHKPSNTKVDKRVESKYGPPCPPCPAPEFLGGPSVFLFPPKPKDTLMISRTPEVTCVVVDVSQEDPEVQFNWYVDGVEVHNAKTKPREEQFNSTYRVVSVLTVLHQDWLNGKEYKCKVSNKGLPSSIEKTISKAKGQPREPQVYTLPPSQEEMTKNQVSLTCLVKGFYPSDIAVEWESNGQPENNYKTTPPVLDSDGSFFLYSRLTVDKSRWQEGNVFSCSVMHEALHNHYTQKSLSLSLGK

SEQ ID NO: 95 - protein, 304 aa, artificial
  amino acid sequence of SEQ ID NO: 85 comprising a glutamic acid at a position corresponding to position 117 of SEQ ID NO: 1
SSPCPQAWGPPGVQYGQPGRSVKLCCPGVTAGDPVSWFRDGEPKLLQGPDSGLGHELVLAQADSTDEGTYICQTLDGALGGTVTLQLGYPPARPEVSCQAADYENFSCTWSPSQISGLPTRYLTSYRKKTVLGADSQRRSPSTGPWPCPQDPLGAARCVVHGAEFWSQYRINVTEVNPLGASTRLLDVSLQSILRPDPPQGLRVESVPGYPRRLRASWTYPASWPCQPHFLLKFRLQYRPAQHPAWSTVEPAGLEEVITDAVAGLPHAVRVSARDFLDAGTWSTWSPEAWGTPSTGHHHHHHHH

SEQ ID NO: 96 - protein, 304 aa, artificial
  amino acid sequence of SEQ ID NO: 85 comprising an arginine at a position corresponding to position 66 of SEQ ID NO: 1
SSPCPQAWGPPGVQYGQPGRSVKLCCPGVTAGDPVSWFRDGEPRLLQGPDSGLGHELVLAQADSTDEGTYICQTLDGALGGTVTLQLGYPPARPVVSCQAADYENFSCTWSPSQISGLPTRYLTSYRKKTVLGADSQRRSPSTGPWPCPQDPLGAARCVVHGAEFWSQYRINVTEVNPLGASTRLLDVSLQSILRPDPPQGLRVESVPGYPRRLRASWTYPASWPCQPHFLLKFRLQYRPAQHPAWSTVEPAGLEEVITDAVAGLPHAVRVSARDFLDAGTWSTWSPEAWGTPSTGHHHHHHHH

SEQ ID NO: 97 - protein, 304 aa, artificial
  amino acid sequence of SEQ ID NO: 85 comprising a serine at a position corresponding to position 65 of SEQ ID NO: 1
SSPCPQAWGPPGVQYGQPGRSVKLCCPGVTAGDPVSWFRDGESKLLQGPDSGLGHELVLAQADSTDEGTYICQTLDGALGGTVTLQLGYPPARPVVSCQAADYENFSCTWSPSQISGLPTRYLTSYRKKTVLGADSQRRSPSTGPWPCPQDPLGAARCVVHGAEFWSQYRINVTEVNPLGASTRLLDVSLQSILRPDPPQGLRVESVPGYPRRLRASWTYPASWPCQPHFLLKFRLQYRPAQHPAWSTVEPAGLEEVITDAVAGLPHAVRVSARDFLDAGTWSTWSPEAWGTPSTGHHHHHHHH

SEQ ID NO: 98 - protein, 304 aa, artificial
  amino acid sequence of SEQ ID NO: 85 comprising a serine at a position corresponding to position 101 of SEQ ID NO: 1
SSPCPQAWGPPGVQYGQPGRSVKLCCPGVTAGDPVSWFRDGEPKLLQGPDSGLGHELVLAQADSTDEGTYICQTLDGASGGTVTLQLGYPPARPVVSCQAADYENFSCTWSPSQISGLPTRYLTSYRKKTVLGADSQRRSPSTGPWPCPQDPLGAARCVVHGAEFWSQYRINVTEVNPLGASTRLLDVSLQSILRPDPPQGLRVESVPGYPRRLRASWTYPASWPCQPHFLLKFRLQYRPAQHPAWSTVEPAGLEEVITDAVAGLPHAVRVSARDFLDAGTWSTWSPEAWGTPSTGHHHHHHHH

SEQ ID NO: 99 - protein, 304 aa, artificial
  amino acid sequence of SEQ ID NO: 85 comprising an serine at a position corresponding to position 178 of SEQ ID NO: 1
SSPCPQAWGPPGVQYGQPGRSVKLCCPGVTAGDPVSWFRDGEPKLLQGPDSGLGHELVLAQADSTDEGTYICQTLDGALGGTVTLQLGYPPARPVVSCQAADYENFSCTWSPSQISGLPTRYLTSYRKKTVLGADSQRRSPSTGPWPCPQDPLGASRCVVHGAEFWSQYRINVTEVNPLGASTRLLDVSLQSILRPDPPQGLRVESVPGYPRRLRASWTYPASWPCQPHFLLKFRLQYRPAQHPAWSTVEPAGLEEVITDAVAGLPHAVRVSARDFLDAGTWSTWSPEAWGTPSTGHHHHHHHH

SEQ ID NO: 100 - protein, 400 aa, Homo sapiens
SSPCPQAWGPPGVQYGQPGRSVKLCCPGVTAGDPVSWFRDGEPKLLQGPDSGLGHELVLAQADSTDEGTYICQTLDGALGGTVTLQLGYPPARPVVSCQAADYENFSCTWSPSQISGLPTRYLTSYRKKTVLGADSQRRSPSTGPWPCPQDPLGAARCVVHGAEFWSQYRINVTEVNPLGASTRLLDVSLQSILRPDPPQGLRVESVPGYPRRLRASWTYPASWPCQPHFLLKFRLQYRPAQHPAWSTVEPAGLEEVITDAVAGLPHAVRVSARDFLDAGTWSTWSPEAWGTPSTGTIPKEIPAWGQLHTQPEVEPQVDSPAPPRPSLQPHPRLLDHRDSVEQVAVLASLGILSFLGLVAGALALGLWLRLRRGGKDGSPKPGFLASVIPVDRRPGAPNL

SEQ ID NO: 101 - protein, 410 aa, Macaca fascicularis
SSPCPQAWGPPGVQYGQPGRPVMLCCPGVSAGTPVSWFRDGDSRLLQGPDSGLGHRLVLAQVDSPDEGTYVCQTLDGVSGGMVTLKLGFPPARPEVSCQAVDYENFSCTWSPGQVSGLPTRYLTSYRKKTLPGAESQRESPSTGPWPCPQDPLEASRCVVHGAEFWSEYRINVTEVNPLGASTCLLDVRLQSILRPDPPQGLRVESVPGYPRRLHASWTYPASWRRQPHFLLKFRLQYRPAQHPAWSTVEPIGLEEVITDTVAGLPHAVRVSARDFLDAGTWSAWSPEAWGTPSTGLLQDEIPDWSQGHGQQLEAVVAQEDSLAPARPSLQPDPRPLDHRDPLEQVAVLASLGIFSCLGLAVGALALGLWLRLRRSGKEGPQKPGLLAPMIPVEKLPGIPNLQRTPENFS

SEQ ID NO: 102 - protein, 401 aa, Mus musculus
SPCPQAWGPPGVQYGQPGRPVMLCCPGVSAGTPVSWFRDGDSRLLQGPDSGLGHRLVLAQVDSPDEGTYVCQTLDGVSGGMVTLKLGFPPARPEVSCQAVDYENFSCTWSPGQVSGLPTRYLTSYRKKTLPGAESQRESPSTGPWPCPQDPLEASRCVVHGAEFWSEYRINVTEVNPLGASTCLLDVRLQSILRPDPPQGLRVESVPGYPRRLHASWTYPASWRRQPHFLLKFRLQYRPAQHPAWSTVEPIGLEEVITDTVAGLPHAVRVSARDFLDAGTWSAWSPEAWGTPSTGLLQDEIPDWSQGHGQQLEAVVAQEDSLAPARPSLQPDPRPLDHRDPLEQVAVLASLGIFSCLGLAVGALALGLWLRLRRSGKEGPQKPGLLAPMIPVEKLPGIPNL

SEQ ID NO: 103 - protein, 6 aa, Artificial Sequence
  8E2 L1 consensus sequence
  VARIANT (3)..(3): X=Y or I or K or M or Q or G or H
VSXYVE

SEQ ID NO: 104 - protein, 6 aa, Artificial Sequence
  8E2 L3.1 consensus sequence
  VARIANT (3)..(3): X=A or H or F or N or S or W
QQXESQ

SEQ ID NO: 105 - protein, 6 aa, Artificial Sequence
  8E2 L3.2
  VARIANT (4)..(4): X=A ow W or T or M or Q or W
ETQXPF

SEQ ID NO: 106 - protein, 6 aa, Artificial Sequence
  8E2 H1 consensus sequence
WWWSIT

SEQ ID NO: 107 - protein, 6 aa, Artificial Sequence
  8E2 H2 consensus sequence
VPWGDL

SEQ ID NO: 108 - protein, 6 aa, Artificial Sequence
  8E2 H3.1 consesnsus sequence
  VARIANT (6)..(6): X=M or R or L
PEDWGX

SEQ ID NO: 109 - protein, 6 aa, Artificial Sequence
  8E2 H3.2 consensus sequence
WGSFWY

SEQ ID NO: 110 - protein, 178 aa, artificial
  Human PAIDY & W147A IL-11 Mutein
PGPPPGPPRVSPDPRAELDSTVLLTRSLLADTRQLAAQLRDKFPADGDHNLDSLPTLPAIDYALGALQLPGVLTRLRADLLSYLRHVQWLRRAGGSSLKTLEPELGTLQARLDRLLRRLQLLMSRLALPQPPPDPPAPPLAPPSSAAGGIRAAHAILGGLHLTLDWAVRGLLLLKTRL